European Patent Application EP 4 782 535 A1, published July 29, 2026. Title: Method for producing regulatory T cells. Applicant: 国立大学法人　大阪大学. The sequence listing filed with the application follows.

SEQUENCE LISTING (16 sequences)

SEQ ID NO: 1 - DNA, 16 bp, synthetic construct
  source 1..16: mol_type = other DNA
cggactgtgaattctt

SEQ ID NO: 2 - DNA, 16 bp, synthetic construct
  source 1..16: mol_type = other DNA
gttgccatagaacatc

SEQ ID NO: 3 - RNA, 20 nt, synthetic construct
  source 1..20: mol_type = other RNA
gaagaattcacagtccgaga

SEQ ID NO: 4 - RNA, 20 nt, synthetic construct
  source 1..20: mol_type = other RNA
agatacttgcatgtagaagg

SEQ ID NO: 5 - DNA, 25 bp, synthetic construct
  source 1..25: mol_type = other DNA
ttgggttaagtttgttgtaggatag

SEQ ID NO: 6 - DNA, 25 bp, synthetic construct
  source 1..25: mol_type = other DNA
atctaaaccctattatcacaacccc

SEQ ID NO: 7 - RNA, 23 nt, synthetic construct
  source 1..23: mol_type = other RNA
gctgcaccggcacattatgatgg

SEQ ID NO: 8 - RNA, 23 nt, synthetic construct
  source 1..23: mol_type = other RNA
aacggaggcgaaaggaacagagg

SEQ ID NO: 9 - RNA, 23 nt, synthetic construct
  source 1..23: mol_type = other RNA
ggaacacggccgcaactggtcgg

SEQ ID NO: 10 - RNA, 23 nt, synthetic construct
  source 1..23: mol_type = other RNA
agaaggctgaagctgcacatcgg

SEQ ID NO: 11 - RNA, 23 nt, synthetic construct
  source 1..23: mol_type = other RNA
gtaatgcaggaccaggctatggg

SEQ ID NO: 12 - RNA, 23 nt, synthetic construct
  source 1..23: mol_type = other RNA
gacgtgggcaacttccactacgg

SEQ ID NO: 13 - protein, 500 aa, Homo sapiens
MDHTEGSPAEEPPAHAPSPGKFGERPPPKRLTREAMRNYLKERGDQTVLILHAKVAQKSYGNEKRFFCPPPCVYLMGSGWKKKKEQMERDGCSEQESQPCAFIGIGNSDQEMQQLNLEGKNYCTAKTLYISDSDKRKHFMLSVKMFYGNSDDIGVFLSKRIKVISKPSKKKQSLKNADLCIASGTKVALFNRLRSQTVSTRYLHVEGGNFHASSQQWGAFFIHLLDDDESEGEEFTVRDGYIHYGQTVKLVCSVTGMALPRLIIRKVDKQTALLDADDPVSQLHKCAFYLKDTERMYLCLSQERIIQFQATPCPKEPNKEMINDGASWTIISTDKAEYTFYEGMGPVLAPVTPVPVVESLQLNGGGDVAMLELTGQNFTPNLRVWFGDVEAETMYRCGESMLCVVPDISAFREGWRWVRQPVQVPVTLVRNDGIIYSTSLTFTYTPEPGPRPHCSAAGAILRANSSQVPPNESNTNSEGSYTNASTNSTSVTSSTATVVS

SEQ ID NO: 14 - protein, 500 aa, Homo sapiens
MDHTEGSPAEEPPAHAPSPGKFGERPPPKRLTREAMRNYLKERGDQTVLILHAKVAQKSYGNEKRFFCPPPCVYLMGSGWKKKKEQMERDGCSEQESQPCAFIGIGNSDQEMQQLNLEGKNYCTAKTLYISDSDKRKHFMLSVKMFYGNSDDIGVFLSKRIKVISKPSKKKQSLKNADLCIASGTKVALFNRLRSQTVSTRYLHVEGGNFHASSQQWGAFFIHLLDDDESEGEEATVRDGYIHYGQTVKLVCSVTGMALPRLIIRKVDKQTALLDADDPVSQLHKCAFYLKDTERMYLCLSQERIIQFQATPCPKEPNKEMINDGASWTIISTDKAEYTFYEGMGPVLAPVTPVPVVESLQANGGGDVAMLELTGQNFTPNLRVWFGDVEAETMYRCGESMLCVVPDISAFREGWRWVRQPVQVPVTLVRNDGIIYSTSLTFTYTPEPGPRPHCSAAGAILRANSSQVPPNESNTNSEGSYTNASTNSTSVTSSTATVVS

SEQ ID NO: 15 - RNA, 20 nt, synthetic construct
  source 1..20: mol_type = other RNA
gtaatgcaggaccaggctat

SEQ ID NO: 16 - RNA, 20 nt, synthetic construct
  source 1..20: mol_type = other RNA
gacgtgggcaacttccacta